European Patent Application EP 4 474 479 A1, published December 11, 2024. Title: DNA-BINDING PROTEIN-A MODULATOR FOR THE TREATMENT OF RENAL ISCHEMIA/REPERFUSION INJURY. Applicant: Otto-von-Guericke-Universität Magdeburg. Application EP. The sequence listing filed with the application follows.

SEQUENCE LISTING (19 sequences)

SEQ ID NO: 1 - RNA, 23 nt, Mus musculus
  source 1..23: mol_type = other RNA
caacggaatcccaaaagcagctg

SEQ ID NO: 2 - DNA, 24 bp, synthetic construct
  source 1..24: mol_type = other DNA
agagaggtatcctgaccctgaagt

SEQ ID NO: 3 - DNA, 24 bp, synthetic construct
  source 1..24: mol_type = other DNA
cacgcagctcattgtagaaggtgt

SEQ ID NO: 4 - DNA, 21 bp, synthetic construct
  source 1..21: mol_type = other DNA
atgtgggaactccggtccata

SEQ ID NO: 5 - DNA, 19 bp, synthetic construct
  source 1..19: mol_type = other DNA
acggcaatctggagcacag

SEQ ID NO: 6 - DNA, 35 bp, synthetic construct
  source 1..35: mol_type = other DNA
tgctctacctggagttcctgcagaagtttgagaag

SEQ ID NO: 7 - DNA, 35 bp, synthetic construct
  source 1..35: mol_type = other DNA
tcatgctctgcggaatgcgcttcagcatctctttc

SEQ ID NO: 8 - DNA, 23 bp, synthetic construct
  source 1..23: mol_type = other DNA
agcaaagaggcctaattgaagtc

SEQ ID NO: 9 - DNA, 20 bp, synthetic construct
  source 1..20: mol_type = other DNA
gaagtagccacagggttggg

SEQ ID NO: 10 - DNA, 20 bp, synthetic construct
  source 1..20: mol_type = other DNA
tgaacggctaaacgagggtc

SEQ ID NO: 11 - DNA, 21 bp, synthetic construct
  source 1..21: mol_type = other DNA
agctccatagggtcttctcgt

SEQ ID NO: 12 - DNA, 20 bp, synthetic construct
  source 1..20: mol_type = other DNA
cagtcccctccctaggactt

SEQ ID NO: 13 - DNA, 20 bp, synthetic construct
  source 1..20: mol_type = other DNA
accctggtcggtttgatgtt

SEQ ID NO: 14 - DNA, 20 bp, synthetic construct
  source 1..20: mol_type = other DNA
taatcgcacatggcctcaca

SEQ ID NO: 15 - DNA, 20 bp, synthetic construct
  source 1..20: mol_type = other DNA
gaagtcctcgggccatgatt

SEQ ID NO: 16 - DNA, 18 bp, synthetic construct
  source 1..18: mol_type = other DNA
ccgcgaagcagcaaccat

SEQ ID NO: 17 - DNA, 20 bp, synthetic construct
  source 1..20: mol_type = other DNA
ccaggtctacgaacactgcc

SEQ ID NO: 18 - DNA, 22 bp, synthetic construct
  source 1..22: mol_type = other DNA
cagactcagaaaatgaagggca

SEQ ID NO: 19 - DNA, 22 bp, synthetic construct
  source 1..22: mol_type = other DNA
agatgggcaagattctcaagtc